European Patent Application EP 4 696 784 A1, published February 18, 2026. Title: MICROORGANISMS FOR PRODUCING GLUTAMATE FAMILY AND PROCESS FOR PRODUCING GLUTAMATE FAMILY USING THE SAME. Applicant: 씨제이제일제당 (주). Application KR. The sequence listing filed with the application follows.

SEQUENCE LISTING (16 sequences)

SEQ ID NO: 1 - protein, 311 aa, Corynebacterium sp.
MNHTLRTLGWLAAVIQEDPEPWFTTDPDTDYVPYVNSFSFESLSLVPDALMLLKRSLHLAMEQQDLPVKDLQEALRHVLVFKFHFREEWELELAWDSERTRSAVETIEYTKDALAEEYQDYKYAFLPELVFQESRGIFEFELEGYTLKVGRGTLSVPWEMVATGYIPASLQNFGELLDADTRDLDADPLLKPRELIFEIHDSEGFDPWIRRETFDFMMGIATEVGWFHSLHPSLNNILVFDLVSRMPGFHIENNFHPHPPNTSWAKLQKIARVVEESEIHSFNMDVLEARYQRFQKLLSPTPVEEPSESST

SEQ ID NO: 2 - DNA, 936 bp, Corynebacterium sp.
  source 1..936: mol_type = genomic DNA
atgaaccacacactccgaacacttggctggcttgctgccgtaattcaagaagatccagagccctggttcaccactgatcccgacaccgattatgtcccttatgtaaatagtttctcatttgaatccctttccctcgttccagatgctctgatgctgctcaaacgttctcttcaccttgcgatggagcaacaggacctcccagtgaaggatctacaagaagcactgaggcacgtactagttttcaaattccacttcagggaagaatgggagctggaattagcatgggactccgagcggacaaggtctgcagtagaaaccattgaatatacaaaagacgcacttgccgaagagtaccaagactacaaatacgcattcttacccgagttagttttccaggaatctcgtggaatctttgagtttgaacttgagggatacacactcaaagtagggcgcggcacgctttcagttccatgggagatggtcgctactggttatatccccgcaagcctccaaaattttggagaactcttggacgcagacaccagagacctagacgcagatcccctcttgaaaccacgggaactcatttttgagattcatgactccgaaggttttgatccttggatacgccgagagacctttgatttcatgatgggtatcgcaaccgaagtcggctggtttcattccctccatccaagcttgaacaatatccttgtcttcgacctagtatcccgcatgcctggattccacatcgagaataatttccatccccacccacccaacacctcctgggcaaagcttcaaaaaattgcccgagtggtggaagaaagcgaaattcattcattcaatatggatgtcctcgaggctcgatatcaaagatttcaaaagttactcagcccaacgccggttgaagaacctagcgagtccagcacataa

SEQ ID NO: 3 - DNA, 34 bp, synthetic construct
  source 1..34: mol_type = other DNA
tcggtacccggggatccgctctagcgtgattgtg

SEQ ID NO: 4 - DNA, 34 bp, synthetic construct
  source 1..34: mol_type = other DNA
gcgcggtttttgtctttgtccattcttatcaatc

SEQ ID NO: 5 - DNA, 34 bp, synthetic construct
  source 1..34: mol_type = other DNA
aaagacaaaaaccgcgcctgcccactactttaat

SEQ ID NO: 6 - DNA, 34 bp, synthetic construct
  source 1..34: mol_type = other DNA
tgcaggtcgactctagaggtggcgtcgagcacgc

SEQ ID NO: 7 - DNA, 20 bp, synthetic construct
  source 1..20: mol_type = other DNA
tattacgccagctggcgaaa

SEQ ID NO: 8 - DNA, 20 bp, synthetic construct
  source 1..20: mol_type = other DNA
gctttacactttatgcttcc

SEQ ID NO: 9 - DNA, 36 bp, synthetic construct
  source 1..36: mol_type = other DNA
cggtacccggggatccctcgtgcggaattcgtggag

SEQ ID NO: 10 - DNA, 20 bp, synthetic construct
  source 1..20: mol_type = other DNA
atccagcagcaattcagaca

SEQ ID NO: 11 - DNA, 37 bp, synthetic construct
  source 1..37: mol_type = other DNA
ctgaattgctgctggattaaggcatcgatatcaccca

SEQ ID NO: 12 - DNA, 36 bp, synthetic construct
  source 1..36: mol_type = other DNA
atgcctgcaggtcgacccttcattttaagttccttg

SEQ ID NO: 13 - DNA, 33 bp, synthetic construct
  source 1..33: mol_type = other DNA
cggtacccggggatccttcatcgatagggtggg

SEQ ID NO: 14 - DNA, 34 bp, synthetic construct
  source 1..34: mol_type = other DNA
gtactcctcagcttactcatcctttgcatcaaca

SEQ ID NO: 15 - DNA, 34 bp, synthetic construct
  source 1..34: mol_type = other DNA
agtaagctgaggagtactgcctgccaaccatcaa

SEQ ID NO: 16 - DNA, 34 bp, synthetic construct
  source 1..34: mol_type = other DNA
atgcctgcaggtcgaccgactggcttgccaccct